European Patent Application EP 4 807 014 A1, published September 16, 2026. Title: ENZYME FOR SYNTHESIZING GLABRIDIN. Applicant: Tsinghua University. The sequence listing filed with the application follows.

SEQUENCE LISTING (39 sequences)

SEQ ID NO: 1 - protein, 353 aa, Pueraria montana var. lobata
MGSNNGRKASEIFQGQALLYRHMFAFVDSMCLKSIVELGIPNIIHKHGQPITLSELMSILQVPPAKVGHVQSLMRYLAHHGFFERLRIHEKDAYALTAASELLVKGTEPYLAPMVECMLDPTLSASFHQMKKWVYEEDLSVFDISLGSNLWDFLTKNPAYNEIFNEAMASDSQMSNLALRDCKLVFEGLESIVDVGGGTGTTAKIICEAFPNLKCIVFDRPQVVENLLENNNLTYVGGDMFKSIPKANAVLLKWILHDWTDKDCRKILENCKEAISNNSKRGKIIIIDIVINEKQDEHKVTELKLLFDVAMACVLNGKERNEEEWKKLFMEVGLQDYKISPLTGYLSLIEIYP

SEQ ID NO: 2 - protein, 366 aa, Glycyrrhiza glabra L.
MDFSTNGSEESELYHAQIHLYKHVYNFVSSMALKSAMELGIADVIHNHGKPITLPQLASALKLHPSKVGVLYRFLRLLTHNGFFAKTTVPSQNGKEGEEEETAYALTPPSKLLVKGKPTCLASIVRGALHPSSLDMWRSSEKWFNEDKELTLFESATGESFWDFLNKDSESGTLSMFQEAMAADSQMFKLALKECRHVFEGLESLVDVGGGTGGVTKLIHEEFPHLKCTVFDQPQVVGNLSGNENLKFVGGDMFKSIPPADAVLLKWVLHDWNDELSLKILKNSKEAISGKGKEGKVIIIDISIDEASGDRELTELQLDYDLVMLTMFNGKEREKKEWEKLISDAGFSSYKITPICGFKSLIEVFP

SEQ ID NO: 3 - protein, 499 aa, Glycyrrhiza echinata
MEILSLLSYSVFYLALFFIFNIVIRARKFKNLPPGPPSLPIIGNLHHLKRPLHRTFKGLSEKYGHVFSLWFGSRLVVVVSSASEFQQCFTKNDVVLANRPRFLSGKYIFYNYTTLGSTSYGEHWRNLRRITALDVLSNHRINSFSGIRRDETQRLITRLADDSSTNFAEMELSSRLYDMTFNNIMRMISGKRYYGEDCDTSDLQEASQFRDMVSELLQLSGANNKTDFMPLLRFLDFENLEKRLKDISGKTDAFLRGLIEEHRTKKERANTMIDHLLNLQDSQPEYYTDQIIKGLALAMLLAGTDSSAVTLEWSMSNLLNHPEVLKKVKDELDTHVGQDRLVDESDLPKLTYLKNVINETLRLYTPAPLLLPHSTSDECNIGGYKVPQDTIVLINAWAIHRDPELWTEATTFKPERFEKKGELEKLIAFGMGRRACPGEGLAIRAISMTLALLIQCFDWKLINGDKIDLAERDGFTLTKLVPLKAMCKSRPVINKVFKQ

SEQ ID NO: 4 - protein, 506 aa, Glycyrrhiza glabra L.
MEILSLLSYSVFYVALFFICNLLFQARKFKNLPPGPPSLPIIGNLHHLKRPLHRTFKGLSEKYGHVISLWFGSRLVVVVSSLSVFQECFTKNDIVLADRPRFLSGKYIFYNYTTVGSSSYGEHWRNLRRITSLDVLSTHRINSFSGVRRDETQRLIQKLAEESSTDFAEIELTSKFYDMTFNNIMRMISGKRYYGDDCDMMDMEEAKQFRAMVSELLQLSGANNKTDFMPVLRLVDFENLEKRLKKISSKTDTFLRGLIQEHRNKKQHTNTMVDHLLSLQESQPEYYTDQIIKGLALGMLLAGTDSSAVTLEWALSCLLNHPEALKKARDELETHVGQDRLLEESDLTKLPYLKNIIYETLRLYTPAPLLLPHSSSDECIIGGFKVPRETIILINAWSIHRDPQIWSEATSFKPERFEKEGELDKLIAFGLGRRACPGEALALRGISLTLGLLIQCFEWKLVGDKEIDMREESGFTLSRLIPLKAMCKARPVANKLVNTQAVSLGD

SEQ ID NO: 5 - protein, 318 aa, Medicago sativa L.
MATENKILILGPTGAIGRHIVWASIKAGNPTYALVRKTPGNVNKPKLITAANPETKEELIDNYQSLGVILLEGDINDHETLVKAIKQVDIVICAAGRLLIEDQVKIIKAIKEAGNVKKFFPSEFGLDVDRHDAVEPVRQVFEEKASIRRVIEAEGVPYTYLCCHAFTGYFLRNLAQLDATDPPRDKVVILGDGNVKGAYVTEADVGTFTIRAANDPNTLNKAVHIRLPKNYLTQNEVIALWEKKIGKTLEKTYVSEEQVLKDIQESSFPHNYLLALYHSQQIKGDAVYEIDPAKDIEASEAYPDVTYTTADEYLNQFV

SEQ ID NO: 6 - protein, 376 aa, Glycyrrhiza glabra L.
MNMIEVGGYPGNPINTKQSNAQQHKPTASLTTYQNKKKKNTHPSFFNSPYFYFNFNIPMAAENKILILGPTGAIGRHIVWASVKAGNPTFALVRKTNGPVNKPKLITAANPESKEQLLESYQNAGVTLLEGDINDHESLVKAIKQVDVVICATGRLLIDDQVKIIAAIKEAGNVKRFFPSEFGLDVDRHDSVEPVREVFEDKARIRRVIEAEGVPYTYLCCHAFTGYFLRNLAQLDATVPPRDKVVILGDGNVKGAYVTEADVGTYTIRAANDPRTLNKAVHIRLPANYLTANEVVSLWEKKIGKTLEKTYVPEEKVLKDIQESSFPHNYLLALYHSQQIKGDAVYEIDPAKDVEAYDLYSDVKYTTADEYLNQFV

SEQ ID NO: 7 - protein, 326 aa, Medicago sativa L.
MAEGKGRVCVTGGTGFLGSWIIKSLLENGYSVNTTIRADPERKRDVSFLTNLPGASEKLHFFNADLSNPDSFAAAIEGCVGIFHTASPIDFAVSEPEEIVTKRTVDGALGILKACVNSKTVKRFIYTSSGSAVSFNGKDKDVLDESDWSDVDLLRSVKPFGWNYAVSKTLAEKAVLEFGEQNGIDVVTLILPFIVGRFVCPKLPDSIEKALVLVLGKKEQIGVTRFHMVHVDDVARAHIYLLENSVPGGRYNCSPFIVPIEEMSQLLSAKYPEYQILTVDELKEIKGARLPDLNTKKLVDAGFDFKYTIEDMFDDAIQCCKEKGYL

SEQ ID NO: 8 - protein, 326 aa, Glycyrrhiza glabra L.
MAEGKGRVCVTGGTGFLGSWLIKRLLEDGYGVNTTIRSDPERKRDISFLTNLPGASERLKIFNADLSDPESFGPAIEGCVGVFHTASPIDFAVSEPEEIVTKRTVDGTLGILKACKNSKTVKRVVYTSSGAAVSWGGTEKDVLDESDWSDVDMLRSVKPYSWSYAVSKTMTEKAVLEFGEQHGLDVVTLILPFIVGRFICPKIPDSVEKALVLVLGKREQIGVTRFHMVHVEDVARAYIFLLEHPNPKGRYNCSPFIVPIEEVSELLSAKYPEYQIPTVEELKEIKGAKLPDLKSKKLVDAGFEFKYTIEDMFDDAIQCCKEKGYL

SEQ ID NO: 9 - protein, 410 aa, Cullen corylifolium
MDWGLAISSSSKAYSVTTGANLWRSKHVTNNIHYPSSCITKASQHKKKTQIEYNVLRFQRPSLGHGYNFSGGGGSTYQECNRKYAVKAVYDQPKDFELEASNPKNILDSAKKFLAAFYYFSYPYTMIGITLCAFCSSALAVEKLSDISLPFFIGVLQAVIPQLFIEIYLSGVNQLYDLEIDKINKPHLPMASGQFSFKTGVIMSAAFLALSFGFTWLTGSWPLIWNLVVIASSWTAYSIDVPFMRWKRYPLVAAMCMIATWGLALPISFFHHMQTFVLQRPIGFPRSLGFLVAFMTFYSMGIALSKDIPDVEGDKEHGINSFSVLLGQKRIFWICVSLFEMAFGVGLLGGVTSPHFWTKIITGLGNVILGSILWYQAKSFDLTDKASTGSFYMYIWKLLYAALLLMAFVR

SEQ ID NO: 10 - protein, 390 aa, Glycyrrhiza glabra L.
MSSLFGSNVFESISTYRSYAPKASQHKRKIQKEYNFLRSRQPSLKHIYKGIEGGSTQQECNRKYVVKTVPKPSFESDPRSIDQKDILECIKNFLDALYMFTTPYSFFSSALYIISVSFIVVEKLSDISPLFFTGVLQAVVPNLFVHIYMTGLNQLCDVEIDKINKPYLPLVSGKISFATGVIVVASCLFLSLWLGWIVGSWPSTCVVISIAMIWTAYSINVPLLRWKKYPVLAAMCIFLSLAVVNPIGYFLHMQTFVFKRPASFSRPLIFVIAFKSFFSLAVALFKDVPDIEGDQTFGVQSFVARFGKKRVFWICISLIEMAYGFALLMGATSAFLWSKIVTVLGHAVLASFVLYRAKSIDLRSKTSITSFYMLIWKLMYMEYFLMPLVR

SEQ ID NO: 11 - protein, 312 aa, Glycyrrhiza glabra L.
MAETTTSKSKILFIGGTGYIGKFIVEASVNAGHPTFVLIRDSTLSNPAKSPIIDKFKSLAVNLVFGDLYDHQSLVKAIKQVDVVISTVGHLQLGDQDKIISAIKESGNVKRFFPSEFGNDVDRTHAVEPAKSAFATKAKIRRTIEAEGIPYTYVSSNFFAGYFLPTLSQPGATAAPRDKVIILGDGNPKAVANKEEDIATYTIKAVDDPRTLNKILYIRPPANTLSFNELVSLWEKKIGKTLGRVYVPEEQLLKQIQESSPPINVILSIGHSVYVKGDHTNFEIEPAFGVEASALYPDVKYTTVDEYLNQFV

SEQ ID NO: 12 - protein, 329 aa, Glycyrrhiza glabra L.
MDSTAASKILVIGGTGYMGRFLVEASAKAGHPTFALVRHSTVTNPDKSSIIHSFNTLGVNLLLGDINDHQSLVKAIKQADVVISTVNHQYISDQYKIISAIKEAGNIKRFFPSEFGNDVVRTHGVDGAKALFDIKAKFRRTIEAEGIPHTYVVANFLTQHFLPTRSRLLAIAAPLDKVVILGDGNTKATFNTEEGVATFTIRAVDDPRTLNKILYIRPPANTLSYNDLVSLWEKKTGNTLERVYVPEEQVLRLIQESSYPLNMALSICHAAYVKGDHTNYEIEPSFGVEALELYPDVKFTTVDDYLEQNRDCTPFYLNQLIPITNGTKF

SEQ ID NO: 13 - protein, 542 aa, Glycyrrhiza glabra L.
MAFTYSTKKLALLSIITIFISSFPEPSTSVDLESGFLQCFSSGLGNSNSTAELVLTKNSSSYASLLQSSIRNLRFMGTSVPKPTLIVTPRDLFHIQTSIKCSVKQGLQIRVRSGGHDYEGLSYVSNDDVPFLIIDLTNLRSITIDIKDETAWVQSGATLGELYYAIAKKSNVHGFPAGSCPTVGVGGHFSGGGFGTIFRKYGLAADNVIDAQMVDVNGKILKNRTLMGEDLFWAIRGGGGSSFGVVTAWKVKLVHVPPKVTVFNIPKTLDQNASTLFHKWQIVADKLPGELFLHSVMGVSNANSISSSSGGGRTVLVSFTGLYLGTVENLLPLMQNNFAELGLQHNNCTEMSWIQSVLFFAGYDPINDSLEVLLQRNQTFGSFKAKSDYVMEPIPTSGLEGLWNMLLEENSSPTLILTPYGGRMSEISESETPFPHRNGSIYGIQYLVYWDSSEETPKHIAWMRRVYSYMVLYVSKFPRAAYLNYRDLDIGVNRGNTSYDYEEAKSWGLKYFKCNFERLAKVKAEVDPSNFFRHEQSIPLLF

SEQ ID NO: 14 - protein, 515 aa, fusarium vanettenii
MLVDTGLGLISELQAKLGWAVLLQIVPITIVAYNLLWFIYASFFSSLRKIPGPFLARISRVWEMKKTATGNIHEIMMDLHRRHGAIVRIGPRRYDFDTMEALKIIYRIGNALPKADYYKPFGLPSFPNLFDEQNPARHSAIKKQVASLYTMTALLSYEEGVDGQTAILKEQLQRFCDQKQVIDLPRFLQYYAFDVIGVITVGKSMGMMESNSDTNGACSALDGMWHYASMMAYIPNMHAWWLRLSSLLPIEVPIKGLTEYVERRIIQYRLKAAEFGDDAALKGENNFLAKLLLMEKKGTVTPVETQQAVGLNIGAGSDTTANALSTILYYLYTNPRTLHTLREELERYVKDGPISFQQSQSMPYLQAVIKEALRLHPGVGTQLTRVVPKGGLVIEGQFFPEGTEVGVNGWALYHNKAIFGNDASIFRPERWLEANENINIGGSFAFGAGSRSCIGKNISILEMSKAIPQIVRNFDIEINHGDMTWKNECWWFVKPEYKAMIKPRRCCLSRDESLV

SEQ ID NO: 15 - protein, 481 aa, Glycyrrhiza glabra L.
MEHFYMSLLLLFVTLVSLSLFFLIFYHNKHNMNNNNNLPPGKMGYPVIGESLEFLSMGWKGHPEKFIFDRMVRYSSELIKTSILGVPTVIFCGPACNKFLFSNENKLVTAWWPDSVNKIFPTTSNSKEESKKMRKLLPQFLKPEALQRYVGIMDTLAQRHFASLWEEKTHVTVYPLAKRYTFMLACRLFMSVEDENHVAKFREPFHLLASGIISVPIDLPWTPFNRGIKASNFIRKELLKIIRQRKVDLAQGVASPTQDILSHMLLTCDDENGEFMTELNIADKILGLLIGGHDTASAACTFIVKYLAELPHIYDRVYQEQMEIANSKSPGELLNWDDINKMRYSWNVASEVMRVAPPLQGGFREAINDFVFNGFSIPKGWKLYWSANSTHKNPEYFPAPEKFDPTRFEGNGPAAYTFVPFGGGPRMCPGKEYARLEILVFMHNLVKRFKWEMLIPEEKIVVDPLPMPANDLPIRLYPHNT

SEQ ID NO: 16 - protein, 369 aa, Cullen corylifolium
ASQHKKKTQIEYNVLRFQRPSLGHGYNFSGGGGSTYQECNRKYAVKAVYDQPKDFELEASNPKNILDSAKKFLAAFYYFSYPYTMIGITLCAFCSSALAVEKLSDISLPFFIGVLQAVIPQLFIEIYLSGVNQLYDLEIDKINKPHLPMASGQFSFKTGVIMSAAFLALSFGFTWLTGSWPLIWNLVVIASSWTAYSIDVPFMRWKRYPLVAAMCMIATWGLALPISFFHHMQTFVLQRPIGFPRSLGFLVAFMTFYSMGIALSKDIPDVEGDKEHGINSFSVLLGQKRIFWICVSLFEMAFGVGLLGGVTSPHFWTKIITGLGNVILGSILWYQAKSFDLTDKASTGSFYMYIWKLLYAALLLMAFVR

SEQ ID NO: 17 - DNA, 1101 bp, synthetic construct
  source 1..1101: mol_type = other DNA
atggacttttcgacaaatgggtctgaggaaagtgaactttatcatgctcaaattcacttgtacaagcatgtttacaattttgtgtcttcaatggctttaaagtcagccatggagttgggcatagctgatgtcatacacaatcatggtaagccaatcaccctcccccagctggcatctgctctgaaattgcacccttctaaggttggagtactttaccgattcctccggttgctaactcacaacggcttctttgctaaaaccactgttccttctcagaatggaaaagaaggcgaggaggaggaaacggcttatgcattgactccaccatcaaaattattggtaaaaggaaagcctacttgtttggcgagcattgttagaggtgcactgcatcctagtagccttgacatgtggagaagttccgagaagtggttcaatgaagataaagagcttacgttattcgagtcagccacaggagaaagtttttgggatttcttgaacaaggacagcgaatcaggaactctctcaatgtttcaagaagcaatggcagcagactctcaaatgttcaaacttgccttgaaggaatgcaggcatgtgtttgagggtttggaatctcttgttgatgtgggtggaggaactggaggggttaccaagttaatccatgaagaatttccccatctgaaatgcacagtatttgatcaaccgcaagtagtggggaacctaagtggaaatgagaatctgaagtttgttggtggtgatatgtttaagagtataccacctgctgatgctgtcctactgaaatgggttcttcatgattggaatgatgagcttagcctcaaaatccttaaaaactccaaggaggctatttctggtaaaggcaaagaagggaaagtgataatcattgacatatcgattgatgaagcgtcaggggatagggaacttacagaattgcagttggattatgatctagtgatgctgacaatgttcaatggtaaggagcgtgagaaaaaggaatgggaaaagctcattagtgacgcaggattttcctcatataaaattacaccaatttgtggtttcaaatctttaattgaggtctttccttga

SEQ ID NO: 18 - DNA, 1521 bp, synthetic construct
  source 1..1521: mol_type = other DNA
atggaaatattgtcactattaagttatagcgtgttctacgtggccctgtttttcatctgcaacctgttgttccaagctcgcaaattcaaaaacctgccaccgggtccgccaagcctgcctatcatcggtaatcttcaccatctgaagcgtccgctgcaccgcaccttcaagggtttgtccgaaaagtacggccacgtgattagcttatggtttggcagccggctggtcgttgttgtgagcagcctgtctgtttttcaggagtgcttcaccaagaacgatattgttttggcggatcgtccgcgtttcctgtctggcaaatacattttttacaattatacgaccgtaggttctagcagctatggcgaacattggcgtaacttgcgccgtatcaccagcctggatgttctttccacccaccgcattaatagcttcagcggtgttcgtcgtgacgaaacgcagcgtttgatccagaaactggcggaggagtcctcgaccgacttcgccgaaattgaattgacttcgaagttttatgatatgaccttcaacaacatcatgcgcatgatctccggcaaacgttattacggcgacgactgtgatatgatggatatggaagaggcgaaacagtttcgtgctatggtgtcagaactcttgcaactgagcggtgcaaataacaagaccgacttcatgccggtcctgcgtctggtggatttcgaaaacctggaaaagcgcctgaagaagatcagcagcaaaaccgacacctttctgagaggcctgatccaagagcaccgcaacaagaagcaacacaccaataccatggttgaccacctgctgtccctgcaagagtctcagccggagtactacactgaccagattatcaaaggtttagcgttaggtatgctgttggcgggcaccgacagctccgcagtcaccttggagtgggcactgagctgcctgctgaatcatccggaggcgcttaagaaggcgcgtgacgagctggaaacgcacgtgggccaggatcgtctcttagaggagtccgacctgacgaaactgccatatctgaagaacattatttacgaaacgctgcgtttatatactccggcaccgctgttgctgccgcattcttcatccgatgaatgtattattggtggttttaaggtgccgcgtgaaaccatcatcctgatcaacgcgtggagcattcatcgtgatccgcagatctggtcggaagctaccagttttaaaccggaacgtttcgagaaggagggtgaactggacaagctgatcgcatttggtctcggtagacgtgcctgcccgggcgaggctttggccctgcgcggtattagcctgacgctgggcctgttgattcaatgttttgagtggaaactggttggtgacaaagaaatcgatatgcgcgaagagagtggctttaccctgagccgtctgatcccgctgaaagctatgtgcaaagctcgcccggttgcgaacaaactggtaaatacccaggcggtgtccctcggggattaa

SEQ ID NO: 19 - DNA, 1131 bp, synthetic construct
  source 1..1131: mol_type = other DNA
atgaacatgattgaagtcggtggttacccaggtaacccaattaacaccaaacaatctaatgcccaacaacacaagccaaccgctagcttgactacttaccaaaacaagaagaaaaagaacactcatccatccttctttaactctccatacttctacttcaacttcaacatcccaatggctgctgaaaacaagatcctgatcttaggtccaactggtgccattggacgtcatatcgtttgggcttccgttaaagccggtaacccaacctttgctttggttagaaagaccaacggtccagttaacaaaccaaagttgatcactgctgccaatccagaatccaaggaacaattactagaatcttaccaaaacgctggtgtcactttgttggaaggtgacattaatgaccacgaatctttggttaaggctatcaagcaagtcgatgtcgtcatctgtgctaccggtagattattgatcgatgaccaagttaagatcattgcagccatcaaggaagccggtaacgttaagagattcttcccatctgaattcggcttggacgttgacagacacgactctgttgaacctgtccgtgaagtcttcgaagataaggctagaattagaagagttatcgaagctgaaggtgttccatacacttacttatgttgtcacgctttcaccggttactttttgagaaacttggctcaattggatgctactgttcctccaagagacaaggttgttattttgggtgatggtaacgtcaagggtgcttacgttactgaagctgacgttggtacatatactatcagagctgctaacgatccaagaaccttgaacaaggctgttcacattagattgccagctaactatttgaccgccaacgaagttgtctccttgtgggaaaagaagattggtaagaccttggaaaagacctacgtcccagaggaaaaagtcttgaaggacatccaagaatcctctttcccacacaactacttgttggccctataccactctcaacaaattaagggtgacgctgtctacgaaatagacccagctaaggatgtcgaagcttacgacttgtactcagatgtaaagtacaccactgctgatgaatacttgaaccaattcgtctga

SEQ ID NO: 20 - DNA, 981 bp, synthetic construct
  source 1..981: mol_type = other DNA
atggccgagggcaagggccgggtatgtgtcacgggcggcaccggcttcctgggatcgtggctgatcaagcgtttgctcgaggacggctacggcgtcaacaccacgatccggagtgacccggagcgcaagcgggacatcagcttcctcaccaacctgcccggggcgagcgagcggctgaagatcttcaacgccgacctgtccgaccccgaatccttcggccccgcgattgaaggctgcgtgggtgtcttccacaccgcctccccgatcgacttcgccgtctcggagcccgaggagatcgtgaccaagcgcaccgtcgacgggacgctgggcatcctcaaggcctgcaagaactccaagaccgtcaagcgggtcgtgtacacgtccagcggcgccgcggtcagctggggcgggaccgagaaggacgtgctcgacgagagcgactggtcggatgtggacatgctgcgctcggtgaagccgtactcctggtcctacgccgtgagcaagacgatgaccgaaaaggcggtgctggagttcggcgagcagcacggcctggacgtcgtcaccctgatcctgccgttcatcgtcggccgcttcatctgccccaagatccccgactccgtcgagaaggcgctggtcctggtgctcggcaagcgcgagcagatcggcgtgacccggttccacatggtccacgtcgaggacgtggccagggcctacatcttcctgctggagcacccgaacccgaaggggcgctacaactgctcccccttcatcgtgccgatcgaggaggtctcggagctcctctccgcgaagtacccagagtaccagatcccgacggtggaggaactcaaggagatcaagggtgccaagctcccggacctcaaatcgaagaagctggtcgacgcggggttcgagttcaagtacaccatcgaggacatgttcgacgacgccatccagtgctgcaaggagaagggatacctgtaa

SEQ ID NO: 21 - DNA, 1173 bp, synthetic construct
  source 1..1173: mol_type = other DNA
atgtcttctttattcgggtcaaatgtatttgagagtatatcaacatatcgtagctatgctccaaaagccagtcaacataaaaggaagattcagaaagaatataatttccttcgctcccgacagccttcattaaagcacatttacaagggaattgagggtggaagtacacaacaagagtgcaataggaaatatgttgtaaaaacagtgcccaagccaagctttgaatcagatcctaggtctatagatcaaaaggacatcttggaatgcattaagaattttcttgatgctttatatatgtttactactccttattcttttttctcctcagcgttgtacattatctccgtttctttcatcgttgtggagaagctttccgacataagcccgctgttcttcactggtgtgctccaagcagttgttccaaatctttttgttcacatatacatgacaggactaaaccagctttgtgatgttgaaattgacaagatcaacaaaccctaccttcccctggtctcaggaaaaattagttttgcaaccggggttattgttgtcgcgtcatgcctgttcctatcgctttggcttggatggattgtgggctcttggccatcaacttgtgtcgtgatatctatcgctatgatttggactgcttactctatcaatgtacctctcctcagatggaagaagtatccagtcctggcagcaatgtgtatatttttatctcttgctgtagtgaaccctattggttatttcttgcatatgcaaacatttgtgttcaagagacctgcttcattttcaaggccgctcattttcgtgattgctttcaaaagtttttttagtttggcagtggcattatttaaggatgttcctgatattgaaggtgatcagacctttggcgttcagtcgtttgttgccagatttggaaagaaaagagttttctggatatgtatttctctcatcgaaatggcatatggttttgctttgttaatgggggctacttccgcttttctatggtccaaaatagttacagtattgggccatgctgttcttgccagttttgtactatatagagcaaaaagcattgatttgcgtagcaaaacgagcattacctctttttacatgttgatatggaaactgatgtatatggagtattttttgatgccattggtccggtga

SEQ ID NO: 22 - DNA, 939 bp, synthetic construct
  source 1..939: mol_type = other DNA
atggctgaaacaactacctcaaaatcaaagattcttttcattggaggaactggctacattgggaaatttattgttgaagcttctgttaatgctggtcatccaacttttgtgttaataagagattcaactctgagcaatccagcgaagtctcccataattgataaattcaagagtctcgcagtgaacctcgtttttggggacttgtatgatcaccagagtcttgtgaaagcaatcaaacaagttgatgttgtgatctccaccgttggacatcttcagcttggagatcaagataagataatatcagccattaaagagtctggtaatgttaagaggtttttcccttctgaatttgggaatgatgtcgaccgtacacatgctgtagagcccgctaagtctgcctttgcaaccaaggcaaaaatccgcaggacaatagaggccgagggaattccatacacttacgtatcgtccaacttctttgctggatatttcttgcctactctatctcaacctggtgcaactgccgctccaagagacaaggttataatcttaggggatggaaaccctaaagctgtcgctaacaaggaggaagatattgctacatatacaatcaaggcggtggatgatccaagaacattgaacaaaatactttatattcggccgccggcaaatactttatctttcaatgaattggtgagtctgtgggaaaagaaaattggtaaaactcttggccgagtttatgtgccagaagagcagctcttgaagcagattcaagaatcgagtcctccaattaatgtcatactaagcatcggccactcagtatatgttaaaggtgatcatacaaattttgagattgagcctgcatttggtgtcgaagcatctgcactgtatcctgacgtaaagtacacgacggttgacgaatatttgaatcaatttgtttga

SEQ ID NO: 23 - DNA, 1629 bp, synthetic construct
  source 1..1629: mol_type = other DNA
atggcttttacgtacagtaccaagaaacttgcactgctctcaatcattactattttcatctccagctttcctgaaccatctacatcggttgaccttgagtcaggcttccttcaatgttttagttcaggattgggcaacagtaacagcacagcggagttggtgctaacaaaaaattcttcctcttatgctagcctgcttcagtctagtattagaaacttgcggttcatgggaacatctgtaccgaagcctacattgatagtgactcctagagatctctttcatatccaaacaagcatcaaatgctcagttaaacaaggattacagatccgtgtaaggtccgggggacatgattacgaaggactctcctacgtttctaatgatgatgtgccatttttgataattgatcttactaatctgcgaagtattaccattgacattaaggatgaaaccgcttgggtccaaagtggagccactcttggagagctatattatgcaattgctaagaagtcgaatgttcacggcttccctgctggttcatgccctacggtaggggttgggggccatttttcaggtggtggatttggaactatatttagaaagtacgggctggccgctgataatgtgattgatgctcaaatggtggatgttaatggaaagatacttaagaataggacattgatgggtgaagatttgttttgggcaatacgggggggtggtggctcatcatttggggtcgttactgcttggaaagttaagttagttcatgttcctccaaaagtaactgtcttcaatatccccaaaacactagatcaaaatgcaagcacccttttccacaaatggcaaattgttgcagataaattgccaggagaactattcttgcattccgtgatgggcgtctctaatgccaattctatttcttcttcctcgggtggaggaagaacagtgcttgtcagctttactggattatatctgggaactgttgaaaatctcttacctctaatgcagaacaattttgctgaattgggtcttcaacacaataactgtacagaaatgagttggattcagagcgtacttttctttgcaggatatgatccaatcaacgattctttagaagtactcctgcagaggaaccagacatttggttctttcaaagcaaaaagcgactatgtgatggagcccataccaacttcagggttggagggcctttggaatatgttattggaagagaatagtagtccaactttgattctcacgccatatggtggtaggatgtctgagataagtgagtctgaaactccatttcctcatcgtaatggttcaatttatggtatacagtatcttgtttattgggattcatctgaggaaactcccaagcatattgcatggatgaggagagtttattcttacatggtactttatgtatcaaagtttccgagggcggcttatttgaattacagagacttagacatcggtgttaaccgagggaatacctcctacgactatgaagaagccaaatcgtggggtctgaaatacttcaaatgtaactttgagagattggctaaggtgaaggcagaggttgatccttcaaacttcttccgccatgaacaatccattcctctcctgttttga

SEQ ID NO: 24 - DNA, 1446 bp, synthetic construct
  source 1..1446: mol_type = other DNA
atggagcatttctacatgtctctactacttttgtttgtaacactggtaagcctttctctctttttcttgattttctatcataacaagcacaatatgaataataacaacaatctaccccctgggaagatgggttatcctgttattggagaatctcttgagtttttgtcaatgggatggaaggggcatcctgagaagttcatatttgacaggatggttcgttacagtagtgagttgatcaaaacatcaatcttaggagtcccaactgtgatcttttgtggaccagcttgtaataagttccttttcagtaatgagaacaaattggtcactgcttggtggccagattctgtaaataagatatttcccacgacttcaaatagcaaagaggaatccaagaaaatgcggaaattgcttcctcaatttcttaagcctgaagctttacagaggtatgttggcataatggatactctggctcagcgacattttgctagtttgtgggaggagaaaactcatgttactgtttacccgctggcaaaacggtacacattcatgcttgcttgccgcctattcatgtctgttgaagatgagaatcatgtggcgaagtttcgcgaacctttccacttgcttgcatctggtatcatatcagtcccaattgatctaccatggacaccatttaacagaggcatcaaggcatcaaattttattaggaaggaactgttaaagataattagacagagaaaagtagatttggcccagggcgtagcgtcccctactcaagatattttaagccatatgttgttaacatgtgatgatgaaaacggtgaatttatgacagaattgaatattgctgataaaatactcggtctcctcattggtggtcatgacacagcatctgccgcatgcactttcatcgtgaagtatttggctgaacttccacacatttatgatagagtttatcaagaacaaatggaaatagctaattcaaaatctccaggagagctgcttaattgggatgacattaacaagatgcgttattcatggaacgttgctagcgaagtcatgagggtggcccctcctcttcaagggggttttcgagaagcaattaatgattttgtgttcaatggattttcgattcccaagggttggaaactctattggagtgcaaactccacgcataaaaatcccgagtattttccagccccggagaaattcgatccaaccaggtttgaaggaaatggccctgctgcatacacctttgttccatttggaggagggccaagaatgtgtcctggaaaagaatatgctagattagagatattggtctttatgcataatcttgttaagagattcaaatgggaaatgctaattccagaagaaaaaatcgttgtggacccgttacctatgccagcaaatgacctgcccattcgtctttaccctcacaacacctga

SEQ ID NO: 25 - DNA, 1062 bp, synthetic construct
  source 1..1062: mol_type = other DNA
atgggttccaacaacggtcgtaaagcttctgaaattttccaaggtcaagctttgctatacagacacatgtttgctttcgtcgactccatgtgtttgaagtccattgtcgaattaggtatcccaaacatcattcacaagcatggtcaaccaatcaccttatccgaattgatgtccatcttgcaagtccctccagctaaggttggtcacgttcaatctttgatgagatatctggctcaccacggtttcttcgaaagattgagaattcacgaaaaggatgcttacgctctgactgctgcttccgaattgttagtcaagggtaccgaaccatacttggctccaatggttgaatgtatgttggatccaactttgtctgcttctttccaccaaatgaagaagtgggtttacgaagaagatttgtcagttttcgacatctccttgggttctaatttatgggatttcttgaccaagaacccagcctacaacgaaatcttcaacgaagctatggcttctgattctcaaatgtctaacttggccttgagagattgcaagttagtctttgaaggtttggaatccatcgtggatgtcggtggtggtactggtactacagccaaaattatttgtgaagccttcccaaacttgaagtgtatcgtctttgacagaccacaagttgttgaaaacttgttagagaacaacaacttgacctacgttggtggtgacatgttcaagtctattccaaaggccaacgctgtcttattgaaatggattctacatgactggactgacaaggactgtcgtaagattttggaaaactgtaaggaagctatctctaacaatagtaagagaggtaagatcatcatcattgacattgttatcaacgaaaagcaagacgagcacaaggtcactgaattgaaattgttgttcgatgttgctatggcctgtgttttgaacggtaaggaaagaaacgaagaagaatggaagaagcttttcatggaagttggattgcaagactacaaaatttctccattgaccggttacttgtctttgatagaaatctacccatga

SEQ ID NO: 26 - DNA, 1500 bp, synthetic construct
  source 1..1500: mol_type = other DNA
atggaaattttgtctttgttgtcctactcagttttctatttggctttgttcttcatcttcaacatcgttatcagagctagaaagttcaagaatttgcctccaggtccaccatctttgccaattatcggtaacctccaccacttaaagagaccattgcatagaaccttcaagggtttgagtgaaaagtacggtcacgttttctccttgtggttcggttccagactggtcgtcgttgtctcctccgcctctgaattccaacaatgtttcaccaagaacgatgttgttctagccaacagaccaagattcctaagcggtaaatacattttctacaactacaccactttgggttctacctcttacggcgaacattggagaaacttacgtagaatcactgctttggatgtcttgtccaaccatagaattaactctttctctggtatcagaagagacgaaactcaaagattgatcaccagattagctgatgactcttccaccaacttcgctgaaatggaattgtcttctagattgtacgacatgactttcaacaatatcatgagaatgatctccggtaagagatactatggcgaagactgtgatacttctgacttgcaagaagcttctcaattcagagacatggtttccgaattgttgcaattgtctggtgctaacaacaaaactgatttcatgccattgttgagattcttggacttcgaaaacttggaaaaaagattgaaggacatttctggtaagaccgatgcttttttgagaggattgattgaagaacacagaactaagaaggaaagagccaacaccatgattgaccacttgttaaatttacaagattcccaaccagaatactacaccgaccaaatcatcaagggtttagccttggccatgttgttggctggtactgactcctctgctgtcactttggaatggtccatgtctaacttgttgaaccacccagaagttttgaagaaagttaaggatgaattggacactcacgtcggtcaagatcgtttagtcgacgaatctgatttgccaaagttgacttacttgaagaacgttatcaacgaaaccttaagattatacactccagctccattgttgctgccacactctacttccgatgaatgtaacattggtggttacaaggttcctcaagacaccattgttttgatcaacgcttgggctattcaccgtgatccagaattatggactgaagctaccacatttaagccagaacgttttgaaaagaaaggtgaattggaaaagttgattgctttcggtatgggtagaagagcttgtccaggtgaaggtctagccattcgtgcaatctctatgaccttggctttgttgattcaatgctttgactggaagttaatcaacggtgacaagatcgacttggctgagagagatggtttcactttgaccaaattggtcccattgaaggctatgtgtaagtctcgtccagttattaacaaggtctttaagcaatga

SEQ ID NO: 27 - DNA, 957 bp, synthetic construct
  source 1..957: mol_type = other DNA
atggctaccgaaaacaagatcttgattttgggtccaactggtgccatcggtagacacattgtctgggcttccatcaaggctggtaaccctacctacgccttagtcagaaagaccccaggtaatgttaacaagccaaagttgatcactgctgctaacccagaaaccaaagaagaattgattgacaactaccaatctttgggtgtcatcttgttggaaggtgacatcaacgaccacgaaacattggtcaaggctattaagcaagtcgatattgttatctgtgctgccggccgtttattgatcgaagaccaagtcaagataatcaaagctatcaaggaagcaggtaacgtcaagaagttcttcccatctgaattcggtttagacgttgacagacatgatgctgttgaaccagttagacaagtttttgaagaaaaagcttccattagaagagttattgaagctgaaggtgttccatacacttatttgtgttgtcacgctttcaccggttacttcttgagaaacttggctcaattggacgccaccgaccctccaagagacaaggttgttattttaggtgatggtaacgttaagggtgcttacgttactgaagctgatgttggtacttttactatccgtgctgctaatgacccaaacactttaaacaaagccgtccatatcagattgccaaagaactacttgactcaaaacgaagtcattgctttgtgggaaaagaagattggtaagaccttggaaaagacttacgtctcagaagaacaagttttgaaggatatccaagaatcttctttcccacacaactatctactggctttgtaccactctcaacaaatcaagggtgatgctgtatacgaaattgatccagctaaggacattgaagcctccgaggcttacccagacgtcacctacaccactgccgatgaatacttgaaccaattcgtctga

SEQ ID NO: 28 - DNA, 981 bp, synthetic construct
  source 1..981: mol_type = other DNA
atggccgaaggtaaaggtagagtctgtgtcaccggtggtactggcttcttgggttcctggattataaagtctttattagaaaacggttactccgtcaacaccactatcagagcagatccagagagaaagagagatgtcagtttcttgactaatttgccaggtgcctctgaaaaattgcacttcttcaacgccgacttgtctaacccagattcttttgctgctgctattgaaggttgtgttggtatcttccacactgctagcccaatcgactttgctgtttccgaaccagaagaaatcgttaccaagagaaccgttgacggtgctcttggaatcttgaaagcttgtgttaactctaagactgtcaagcgtttcatttacacctcttctggttctgctgtttctttcaatggtaaggacaaggatgttttggacgaatccgactggtctgacgtcgacttgttgagatctgtcaagccattcggttggaactacgctgtctccaagaccctagctgaaaaggctgtattggaattcggtgaacaaaacggtattgacgttgttactttgattttgcctttcattgtcggtcgtttcgtctgccctaagttgccagactccattgaaaaggctttggtcctagttttgggtaagaaagaacaaattggtgttaccagatttcacatggttcacgttgatgacgtcgccagagcccatatctatttattggaaaactccgttccaggtggtagatacaactgttctccattcatcgttccaattgaagaaatgtcacaattgttgtccgctaagtacccagaataccaaatcttgactgtggatgaattgaaggaaatcaagggtgctagattaccagatttgaacactaagaagttagtcgatgctggtttcgacttcaagtacacaatcgaagacatgttcgatgatgctatccaatgttgtaaggaaaagggttacttgtga

SEQ ID NO: 29 - protein, 1110 aa, synthetic construct
GCATCTCAACACAAGAAGAAGACTCAAATCGAATACAACGTCTTGAGATTCCAAAGACCATCCTTGGGTCACGGATACAACTTCTCCGGTGGTGGTGGCTCCACTTACCAAGAATGTAACAGAAAGTACGCCGTTAAGGCTGTCTACGACCAACCAAAGGACTTCGAATTGGAAGCTTCCAACCCAAAGAACATTTTGGACTCTGCCAAGAAATTCTTGGCTGCTTTTTACTACTTCAGTTACCCATACACCATGATTGGTATCACTTTGTGCGCTTTCTGTTCCTCTGCTTTAGCTGTCGAAAAGTTGTCTGATATCTCCCTCCCTTTCTTCATCGGTGTCTTGCAAGCTGTTATCCCACAATTGTTTATTGAAATTTACTTGTCTGGTGTTAACCAATTATATGACTTGGAAATCGACAAGATTAACAAGCCACATTTGCCAATGGCTTCTGGTCAATTCTCTTTCAAGACCGGTGTCATCATGTCTGCCGCCTTTTTGGCTTTGTCCTTCGGTTTCACCTGGTTGACCGGATCTTGGCCATTGATCTGGAACTTGGTTGTTATTGCCTCCTCCTGGACTGCTTACTCTATTGACGTTCCATTCATGAGATGGAAGAGATACCCATTAGTTGCTGCTATGTGTATGATCGCTACCTGGGGTCTGGCTTTACCAATCTCTTTTTTCCACCACATGCAAACTTTCGTTTTGCAACGTCCTATTGGTTTCCCAAGATCTTTGGGTTTCTTGGTTGCTTTCATGACTTTTTATTCCATGGGTATTGCTTTGAGCAAGGATATTCCAGATGTTGAAGGTGACAAGGAACATGGTATCAATTCTTTCTCAGTCTTGTTGGGTCAAAAGCGTATCTTCTGGATCTGTGTCTCATTGTTTGAAATGGCTTTCGGTGTTGGTCTATTAGGTGGTGTTACTTCTCCACACTTCTGGACCAAGATCATTACCGGTCTAGGTAACGTCATTTTGGGTTCCATCTTGTGGTACCAAGCTAAGTCTTTCGATTTGACAGATAAAGCTTCTACTGGTTCTTTCTACATGTACATCTGGAAATTGTTGTACGCTGCCTTATTGTTGATGGCCTTCGTCAGATGA

SEQ ID NO: 30 - protein, 939 aa, synthetic construct
ATGGCCGAAACCACCACTTCTAAGTCTAAAATATTGTTTATTGGTGGTACCGGTTACATTGGCAAGTTCATTGTTGAAGCCAGTGTCAATGCCGGTCACCCAACTTTCGTCTTGATTAGAGATAGCACTTTGTCTAACCCAGCGAAGTCCCCAATCATTGATAAATTCAAGTCTTTGGCTGTCAACTTGGTTTTCGGTGACTTGTACGACCACCAATCTTTGGTCAAGGCCATCAAACAAGTTGATGTAGTGATCTCCACAGTCGGTCATTTGCAATTGGGTGACCAAGACAAGATTATTTCCGCTATCAAGGAATCCGGTAATGTCAAGAGATTCTTCCCATCAGAATTCGGTAACGACGTTGACAGAACCCACGCTGTCGAACCAGCTAAATCCGCTTTCGCTACCAAGGCTAAGATCAGACGTACTATCGAAGCTGAAGGTATCCCATACACTTACGTTTCTTCCAACTTTTTTGCTGGTTACTTCTTGCCAACCTTATCCCAACCAGGTGCTACTGCTGCTCCAAGAGACAAGGTTATCATCTTGGGTGACGGTAACCCAAAGGCTGTTGCTAACAAGGAAGAAGATATTGCTACTTACACTATCAAGGCAGTCGATGACCCACGTACCTTAAACAAGATTTTGTACATCAGACCACCAGCCAACACTCTATCTTTCAACGAATTGGTTTCCTTATGGGAAAAGAAGATCGGTAAGACCTTGGGTAGAGTCTATGTCCCAGAAGAACAACTGTTGAAGCAAATTCAAGAGTCTTCTCCACCTATCAACGTTATCTTATCTATTGGTCACTCTGTTTACGTCAAGGGTGACCACACCAACTTCGAAATTGAACCTGCTTTCGGTGTTGAAGCCTCTGCTTTGTATCCAGATGTTAAGTACACCACTGTTGATGAATACTTGAACCAATTCGTTTGA

SEQ ID NO: 31 - DNA, 1629 bp, synthetic construct
  source 1..1629: mol_type = other DNA
atggctttcacttactccactaagaagttggctttgttgtctatcatcactatattcatctcctccttcccagaaccatctacttctgttgatttggaatctggtttcttgcaatgtttctcttctggtctaggtaactctaactcaactgctgaattggtcttgaccaagaactcttcctcttacgcctccctgttgcaatcttccattcgtaatctgagattcatgggtacctcggtcccaaagccaaccttgattgtcactccacgggatttgttccatattcaaacctctattaagtgttctgttaagcaaggtttgcaaatcagagttagatcaggtggtcacgactacgaaggtttgtcctacgtctccaacgatgacgttccattcctgattatcgacttgaccaacttgcgtagtatcaccattgacatcaaggacgaaactgcttgggttcaatctggtgcaactttgggtgaattgtactacgctattgccaagaagtctaacgtccacggtttcccagctggttcttgtccaaccgtcggtgttggtggtcacttctctggtggtggtttcggtaccatcttcagaaagtacggtctagccgctgataacgttatcgacgctcaaatggttgatgtcaacggtaagatcttgaagaacagaaccttgatgggtgaagacttgttctgggctatcagaggcggtggtggttcttcctttggtgtcgtcaccgcttggaaggttaaattggtccatgttccaccaaaagtgacagttttcaacatccctaagaccttggaccaaaacgcttctaccttgttccacaagtggcaaatcgttgctgacaagttaccaggtgaattgtttttgcacagtgtcatgggtgtttccaacgccaactccatttcctcatcttccggtggcggtcgtactgtcttagtttctttcaccggcttgtacttgggtactgttgagaacctattgccattgatgcaaaacaactttgctgaattaggtttacaacacaacaactgtactgaaatgtcctggattcaatccgttttattctttgccggttacgacccaatcaacgactctttggaagttttgttacaaagaaaccaaactttcggttccttcaaggccaagtctgactacgttatggaacctattccaactagcgggttggaaggtttgtggaacatgttgctcgaagaaaatagctctccaactttgatcttgactccatacggtggtagaatgtctgaaatttctgaatctgaaaccccgttcccacacagaaatggttccatctacggtatccaatacttagtttactgggattcctccgaagaaaccccaaagcatattgcttggatgagaagagtctactcttacatggttttgtacgtttctaagttcccaagagctgcttacttgaactacagagatttggatattggtgttaacagaggtaacacttcctatgactatgaagaagccaaatcttggggtttaaagtatttcaaatgcaatttcgaaagattggctaaagtcaaggctgaagtcgatccttctaacttcttcagacacgaacaatctattccattgttattttga

SEQ ID NO: 32 - DNA, 1548 bp, synthetic construct
  source 1..1548: mol_type = other DNA
atgctcgttgacactggtttaggattgatttctgaattgcaagccaagttgggttgggctgttttgttgcaaattgtcccgatcaccatcgtcgcttacaacttactgtggttcatctacgcttccttcttttcctctttgagaaagattccaggtccattcttggctcgtatctcccgtgtctgggaaatgaagaagactgctaccggtaacattcacgaaatcatgatggacttgcacagacgtcacggtgctatcgtcagaatcggtccaaggagatatgacttcgacaccatggaagctttgaagatcatttacagaattggtaatgccttgcctaaagctgactactacaagccattcggtttgccatctttcccaaacttgtttgatgaacaaaacccagctagacattccgctatcaagaaacaagttgcttctttgtacactatgactgctttattgtcttacgaagaaggtgtcgatggtcaaaccgccatcttgaaggaacaattgcaaagattctgtgaccaaaagcaagtcattgatttgccaagattcttgcaatactacgctttcgatgttatcggtgttatcactgttggtaagtctatgggtatgatggaatccaactctgatactaatggtgcttgctctgctttggacggtatgtggcactacgcctccatgatggcttacatccctaacatgcacgcttggtggttgagattgagctctcttttgccaatcgaagttccaattaagggtttgactgaatacgttgaaagaagaatcatccaatacagattaaaggctgctgaattcggtgatgatgctgccttgaaaggtgaaaacaactttttggctaagttgttgttgatggaaaagaagggtacagtcactccagtggaaactcaacaagctgtcggcttgaacattggtgctggttctgacactactgcgaacgctttgagtaccatcttgtattatttatacaccaacccaagaaccctgcacactttgagagaagagttggaacgttacgtcaaggatggtccaatctctttccagcaatctcaatccatgccatacttgcaagctgtcatcaaggaagccctaagattacatccaggtgttggtacccaattgaccagagttgttccaaagggtggtttagtcattgaaggtcaattcttcccagaaggtaccgaagtcggtgttaacggttgggctctataccacaacaaggccatttttggtaacgatgcctccatcttcagaccagaaagatggttagaagctaacgaaaacattaacatcggtggttctttcgccttcggtgccggttccagatcttgtatcggcaagaatatcagcattttggaaatgtccaaggctattccacaaattgttagaaacttcgacattgaaattaaccacggtgacatgacctggaagaacgaatgttggtggttcgttaaaccagaatacaaggctatgattaagccaagaagatgttgtttgtctagagacgaatctctggtttga

SEQ ID NO: 33 - DNA, 1101 bp, synthetic construct
  source 1..1101: mol_type = other DNA
atggacttctctaccaacggttctgaagaatcagaattataccacgctcaaatccatttatataagcacgtttacaacttcgtttcttccatggctctgaagtctgctatggaattgggtattgccgatgttattcacaatcacggtaagccaattactttgccacaattggctagtgctttgaagttgcacccatctaaggtcggcgttttatacagattcttgagattattgactcacaatggttttttcgctaagaccactgttccgtcacaaaacggtaaggaaggtgaggaagaagaaaccgcttacgctttgaccccaccttccaaattgttggtcaagggtaagccaacttgtttggcctccattgtcagaggtgctttgcatccaagctctcttgacatgtggagatcttctgaaaagtggtttaacgaagacaaggaattaacattgttcgaatccgccactggtgaatctttctgggatttcttgaacaaggactccgaatctggtactttgtccatgttccaagaagccatggctgctgactctcaaatgttcaagttggccttgaaggaatgtagacacgtctttgaaggtttggaatctttagtcgatgttggtggaggtaccggtggtgtcaccaagttgatccacgaagaattcccacatttgaaatgcaccgtcttcgaccaaccacaagttgttggtaacttgtctggtaacgaaaacctaaaattcgtcggtggtgacatgtttaagtccatcccaccagctgatgctgtcttgttgaaatgggttttgcacgactggaacgatgaactatctttgaagattttgaagaactccaaggaagctatctccggtaagggtaaagaaggtaaggttatcatcattgatatttctatcgacgaagcttccggtgatcgtgaattgactgaattgcaattggactacgatttggttatgttgaccatgttcaacggtaaggaaagagaaaagaaggaatgggaaaaattaatctctgacgctggtttctcctcttacaagatcactccaatctgtggtttcaagtccttgattgaagttttcccatga

SEQ ID NO: 34 - DNA, 1521 bp, synthetic construct
  source 1..1521: mol_type = other DNA
atggaaatcttgtccttgttgtcttactccgttttttacgttgctttgttcttcatctgtaacttgttattccaagctagaaagttcaagaatttgccacctggtccaccatctctcccaatcattggtaacttacatcatttgaagagaccattgcacagaactttcaagggattgtctgaaaagtacggtcacgttatctctttgtggttcggttctagattggttgtcgtcgtgtcttccttatctgtcttccaagaatgcttcaccaagaacgatattgttctcgctgacagaccaagattcttgagtggtaaatatatcttctacaactacaccactgtcggttcctcttcctacggtgaacactggagaaacttaagaagaatcacttccttagatgtcttgtccacccacagaattaactctttctctggtgttagaagagatgaaacccaaagactgatccaaaagttggccgaagaatcatccactgattttgctgaaattgaattgacctccaagttttacgatatgactttcaacaacatcatgagaatgatttccggtaagagatactacggcgatgactgtgacatgatggacatggaagaagctaagcaattcagggccatggtttccgaattgctacaattgtctggtgctaacaacaagaccgacttcatgccagtcttgagattggtcgatttcgaaaacttggaaaaacgtttaaagaagatctcctctaagactgacaccttcttgcgtggtttgatccaagaacacagaaataagaagcaacacaccaacaccatggttgaccacttgctgtctttgcaagaatctcaaccagaatactatactgaccaaatcatcaagggtttagccttgggtatgttgttggctggtaccgattcctcagctgttactttggaatgggctctatcttgtttgttgaaccacccagaagccttgaagaaggcaagagacgaattagaaacccatgtcggtcaagatcgtttgttggaagaatccgatttgacaaaattgccatacttgaagaacattatctacgaaactttgagattgtacactccagctccattattgttgcctcactcttcttctgacgagtgtatcatcggtggtttcaaggttccaagagaaactattattttgattaacgcttggtctattcaccgtgacccacaaatctggtctgaagctacttctttcaagccagaaagatttgaaaaggaaggtgaattggacaaattaattgctttcggtctgggtagaagagcttgtccaggtgaagctttggccttgagaggtatctctttgaccttgggtctattgattcaatgtttcgaatggaagttggttggtgacaaggaaattgacatgcgtgaagaatctggtttcactttatccagattaattccattgaaggctatgtgtaaggctcgtccagttgccaacaaattagttaacactcaagctgtctctttgggtgattga

SEQ ID NO: 35 - DNA, 981 bp, synthetic construct
  source 1..981: mol_type = other DNA
atggctgaaggtaagggtagagtctgtgtcaccggtggtactggtttcctaggttcatggttaatcaagcgtttattggaagacggttacggcgtcaacactaccatcagatccgacccagaaagaaagagagacatttctttcttgactaacttgccaggtgcctccgaaagattaaaaatcttcaatgctgacttgtccgacccagaatccttcggaccagctattgaaggttgtgttggtgtcttccacactgcttccccaattgacttcgccgtcagtgaaccagaagaaattgtcaccaagcgtactgttgatggtactttgggtatcttgaaggcttgcaagaactccaagactgttaagagagttgtctacacctcttctggtgctgctgtctcttggggtggtaccgaaaaggatgtcttggacgaatctgactggtccgatgtggacatgttgagatctgtcaagccatactcttggtcttacgctgtttccaagaccatgactgaaaaggccgtcttggaattcggtgaacaacacggtttggatgttgttacattgattttgccattcattgtcggtagatttatctgtccaaagatccctgactctgttgagaaagctttggtcctcgttttgggtaagagagaacaaatcggtgttaccagattccacatggttcatgttgaagacgttgctagagcttacatctttttgcttgaacacccaaacccaaaggggagatacaactgttctccatttattgttccaatcgaagaagtttctgaattgttgtctgccaaatacccagaataccaaattccaaccgttgaagaattaaaagaaatcaagggtgctaagttgcctgatttgaagtctaaaaagttagttgatgctggtttcgaattcaagtacactattgaagatatgttcgacgatgccatccaatgttgtaaggaaaagggttatttgtga

SEQ ID NO: 36 - DNA, 1173 bp, synthetic construct
  source 1..1173: mol_type = other DNA
atgtcttctctatttggctctaacgttttcgaatccatttccacttacagatcttacgctccaaaggcttctcaacacaagagaaagatccaaaaggaatacaacttcttaagatccagacaaccatctttgaagcacatttacaagggtatcgaaggtggttccactcaacaagaatgtaacagaaagtacgtcgttaagaccgttccaaaaccatcctttgaatctgacccaagatccatcgaccaaaaggatattttggaatgtatcaagaactttttggatgccctttatatgttcaccactccatactcgttcttttcctccgctttgtacatcattagtgtttctttcatcgttgttgaaaagttgtctgacatttccccattgttcttcaccggtgtcttgcaagctgtggttccaaacttgttcgtccatatctacatgacaggtttgaaccaattgtgtgatgtcgaaatcgacaagatcaacaagccttacttgccattggtctctggtaaaatttcctttgccaccggtgtaattgtcgttgcttcttgtctcttcttgtccttgtggttgggttggatcgtcggttcttggccttctacctgtgtcgtcatctccatagccatgatctggactgcttactctatcaatgttccattattgagatggaagaaatacccagttttggctgctatgtgtattttcttgtctttggccgtcgttaacccaattggttacttcttacacatgcaaactttcgtcttcaagcgtccagcttccttctctagaccattgatcttcgttatagctttcaaatctttcttctctttagccgtcgctttattcaaggacgtcccagacattgaaggtgatcaaaccttcggtgtccaatcttttgttgcccgtttcggtaagaagagagttttctggatctgcatcagtttgattgaaatggcttacggtttcgctttgttgatgggtgctacttctgctttcttatggtctaagattgtcactgttttgggtcacgctgttttggcatcattcgttttgtatagagctaagtctattgatttgagatccaagacttccattacctctttctacatgttgatctggaagctaatgtacatggaatacttcttgatgccattagttagatga

SEQ ID NO: 37 - DNA, 990 bp, synthetic construct
  source 1..990: mol_type = other DNA
atggactctactgctgcctccaagatcttggttattggtggtactggttacatgggtcgttttctggtcgaagcttctgccaaggccggtcatcctacctttgctttagtacgtcacagtactgttaccaacccagacaagtcctctattattcactctttcaacaccctaggcgtcaatctattgttgggtgacattaatgatcatcaatctttggtcaaggccatcaagcaagctgatgttgtcatctctaccgttaaccaccaatatatttctgaccaatacaagattattagcgctatcaaggaagcaggtaacatcaaacgtttcttcccatctgaattcggtaacgacgttgtcagaactcacggtgtcgacggtgctaaggctttgttcgatatcaaggctaaattcagaagaaccatcgaagctgaaggtatccctcacacttacgtcgttgccaacttcttgactcaacacttcttgccaactagatccagattattggctattgctgctccattagataaggttgtcatattgggtgatggtaacaccaaggccacattcaacactgaagaaggtgttgctaccttcactatcagagctgtcgacgacccaagaactttgaacaagatcttatacattagaccaccagctaacactttgtcctacaacgatttggtttccttgtgggaaaagaagaccggtaacaccttggaaagagtttatgttccagaagaacaagttttgagattgatccaagaatcttcttacccattgaacatggctttgtccatctgtcacgctgcttacgttaagggtgaccacaccaactacgaaattgaaccatccttcggtgttgaagccttggaattgtacccagatgtcaagttcaccactgtggatgactacttggaacaaaacagagactgtactccattctacttaaatcaattgattccaatcactaacggtaccaaattttga

SEQ ID NO: 38 - DNA, 1629 bp, synthetic construct
  source 1..1629: mol_type = other DNA
atggctttcacttactccaccaagaaattggctttgttgtctattatcaccatcttcatctcctctttcccagaaccatctacctctgttgacttggaatccggtttcctgcaatgtttttccagtggtttgggtaactctaattccactgcagaattggttttgaccaagaactcgtcctcttacgcctccttgttgcaatcctccatccgtaacctaagattcatgggtacttccgtcccaaagccaactttgattgtcactccaagagacttgttccatatccaaacctccatcaaatgcagcgttaagcaaggtttgcaaattcgtgtcagatccggtggtcatgactacgaaggtttatcctacgtctccaacgatgacgttccattcttgattatcgacttgaccaacttgagatccatcactatcgatatcaaggatgaaactgcttgggttcaatctggtgctaccttgggtgaattatattacgctattgctaagaagtctaacgttcacggtttcccagctggttcttgtccaactgtcggtgttggtggtcacttctctggtggtggtttcggtaccattttcagaaagtacggtttagccgctgacaacgtcattgacgctcaaatggttgatgttaacggtaagatcttgaagaacagaactttgatgggtgaagatttgttttgggctatcagaggtggtggtggttcttccttcggtgttgttaccgcttggaaggtcaagttggtccatgttcctccaaaagttactgttttcaacattccaaagaccttggaccaaaatgcttctactttattccacaagtggcaaattgttgctgataagttgccaggtgaattgtttttgcactctgtcatgggtgtctctaacgctaactctatttcttcttcctcaggtggcggtagaaccgtcctagtctctttcaccggtctatacttgggtaccgttgaaaacttgttgccattgatgcaaaacaactttgctgaattaggtttgcaacacaacaactgtactgaaatgtcttggattcaatctgtacttttctttgccggctacgacccaatcaacgacagtttggaggtcttacttcaaagaaaccaaactttcggttctttcaaggccaaatctgactacgttatggaacctatcccaacctctggtttggaaggtttatggaacatgttgttggaagaaaattcttctccaactttgattttgactccatacggtggtagaatgtccgaaatctctgaatctgaaaccccattccctcacagaaacggatccatctacggtatccaatacttggtttactgggattcttctgaagaaacaccaaagcacatcgcctggatgagaagagtctactcttacatggtcttgtacgtttccaagttcccaagagctgcttacttgaactacagagatttggatattggtgtcaaccgtggtaacacttcttatgactatgaagaagctaagtcctggggtctcaaatacttcaagtgtaacttcgaaagattggccaaggttaaggctgaagttgacccatccaacttcttcagacacgaacaatccattccattgttgttttga

SEQ ID NO: 39 - DNA, 1446 bp, synthetic construct
  source 1..1446: mol_type = other DNA
atggaacacttttatatgtctttattgttactattcgttacattggtttctttgagcttattcttcttgatcttttaccacaacaagcacaacatgaacaacaacaacaatttgcctccaggtaagatgggttacccagttatcggtgaatctttggaatttttgtccatgggttggaagggtcaccctgaaaagttcattttcgacagaatggttagatactccagtgagttaattaagacttccatcttgggtgttccaactgtcatcttctgtggtccagcttgtaacaaattcttgttctctaacgaaaataagttggtgactgcttggtggccagactctgtcaacaaaatcttcccaaccacttctaattctaaggaagaatccaagaagatgagaaagttgttgccacaattcttgaagccagaagctttgcaacgttacgttggcattatggacactttagctcaaagacacttcgcgtctttgtgggaagaaaagacccatgtcaccgtttatcctttggctaagagatacactttcatgttggcctgtagattgttcatgtctgttgaagatgaaaaccacgttgccaagttcagagaaccattccatttgttggcctccggtatcatctctgtcccaattgacttgccatggactccattcaacagaggtatcaaggcttcaaacttcatcagaaaagaattgttgaaaattatcagacaaagaaaggtcgacttagctcaaggtgtcgcttccccaacccaagatatcttgtctcacatgttgctcacctgtgatgacgaaaacggtgaattcatgactgaattgaacatcgctgacaagattttgggtttgttgattggtggtcatgacaccgcttccgctgcttgcactttcattgtcaagtacctagctgaacttcctcacatttacgatagagtctaccaagaacaaatggaaattgctaactctaagtctccaggtgaattgctcaactgggatgatatcaacaagatgcgttactcttggaacgttgcttctgaagttatgagagttgccccaccattgcaaggtggtttccgtgaagctattaacgatttcgtctttaatggtttctccataccaaagggttggaagttgtactggtctgccaactccacccacaagaacccagaatacttcccagctccagaaaagtttgacccaaccagattcgaaggtaacggtccagccgcttacaccttcgtcccgttcggtggtggaccaagaatgtgtccaggtaaggaatacgctagattggaaatcctagttttcatgcacaacttggtcaaacgttttaagtgggaaatgttgattccagaagaaaagattgttgtcgatccattgcctatgccagccaacgacctaccaatcagattatacccacacaacacttga